European Patent Specification EP 3 442 602 B1, published February 19, 2025. Title: ADENO-ASSOCIATED VIRUS VECTOR DELIVERY OF MICRODYSTROPHIN TO TREAT MUSCULAR DYSTROPHY. Applicant: RESEARCH INSTITUTE AT NATIONWIDE CHILDREN'S HOSPITAL RODINO-KLAPAC, et al. The sequence listing filed with the application follows.

SEQUENCE LISTING (12 sequences)

SEQ ID NO: 1 - DNA, 5910 bp, Adeno-associated virus
  promoter (120)..(526): CMV promotor
  Intron (927)..(1087): EF1a intron
  misc_feature (1088)..(1375): shRNA-miR29-c
  misc_feature (1257)..(1284): miR-29c
  Intron (1380)..(1854): EF1a intron
  misc_feature (1896)..(2091): polyA
cagcagctgcgcgctcgctcgctcactgaggccgcccgggcaaagcccgggcgtcgggcgacctttggtcgcccggcctcagtgagcgagcgagcgcgcagagagggagtggggttaaactcgttacataacttacggtaaatggcccgcctggctgaccgcccaacgacccccgcccattgacgtcaataatgacgtatgttcccatagtaacgccaatagggactttccattgacgtcaatgggtggagtatttacggtaaactgcccacttggcagtacatcaagtgtatcatatgccaagtacgccccctattgacgtcaatgacggtaaatggcccgcctggcattatgcccagtacatgaccttatgggactttcctacttggcagtacatctacgtattagtcatcgctattaccatggtgatgcggttttggcagtacatcaatgggcgtggatagcggtttgactcacggggatttccaagtctccaccccattgacgtcaatgggagtttgttttggcaccaaaatcaacgggactttccaaaatgtcgtaacaactccgccccattgacgcaaatgggcggtaggcgtgtacggtgggaggtctatataagcagagctcgtttagtgaaccgtcagatcgcctggagacgccatccacgctgttttgacctccatagaagacaccgggaccgatccagcctccggactctagaggatccggtactcgaggaactgaaaaaccagaaagttaactggtaagtttagtctttttgtcttttatttcaggtcccggatccggtggtggtgcaaatcaaagaactgctcctcagtggatgttgcctttacttctaggcctgtacggaagtgttacttctgctctaaaagctgcggaattgtacccggggccgatccaccggtctttttcgcaacgggtttgccgccagaacacaggtaagtgccgtgtgtggttcccgcgggcggcgacggggcccgtgcgtcccagcgcacatgttcggcgaggcggggcctgcgagcgcggccaccgagaatcggacgggggtagtctcaagctggccggcctgtttgaatgaggcttcagtactttacagaatcgttgcctgcacatcttggaaacacttgctgggattacttcttcaggttaacccaacagaaggctcgagaaggtatattgctgttgacagtgagcgcaaccgatttcaaatggtgctagagtgaagccacagatgtctagcaccatttgaaatcggttatgcctactgcctcggaattcaaggggctactttaggagcaattatcttgtttactaaaactgaataccttgctatctctttgatacattggccggcctgctctggtgcctggcctcgcgccgccgtgtatcgccccgccctgggcggcaaggctggcccggtcggcaccagttgcgtgagcggaaagatggccgcttcccggccctgctgcagggagctcaaaatggaggacgcggcgctcgggagagcgggcgggtgagtcacccacacaaaggaaaagggcctttccgtcctcagccgtcgcttcatgtgactccacggagtaccgggcgccgtccaggcacctcgattagttctcgagcttttggagtacgtcgtctttaggttggggggaggggttttatgcgatggagtttccccacactgagtgggtggagactgaagttaggccagcttggcacttgatgtaattctccttggaatttgccctttttgagtttggatcttggttcattctcaagcctcagacagtggttcaaagtttttttcttccatttcaggtgtcgtgaaaagctagcgctaccggactcagatctcgagctcaagctgcggggatccagacatgataagatacattgatgagtttggacaaaccacaactagaatgcagtgaaaaaaatgctttatttgtgaaatttgtgatgctattgctttatttgtaaccattataagctgcaataaacaagttaacaacaacaattgcattcattttatgtttcaggttcagggggaggtgtgggaggttttttcactagtagcatggctacgtagataagtagcatggcgggttaatcattaactacaaggaacccctagtgatggagttggccactccctctctgcgcgctcgctcgctcactgaggccgggcgaccaaaggtcgcccgacgcccgggctttgcccgggcggcctcagtgagcgagcgagcgcgccagctggcgtaatagcgaagaggcccgcaccgatcgcccttcccaacagttgcgcagcctgaatggcgaatggaattccagacgattgagcgtcaaaatgtaggtatttccatgagcgtttttcctgttgcaatggctggcggtaatattgttctggatattaccagcaaggccgatagtttgagttcttctactcaggcaagtgatgttattactaatcaaagaagtattgcgacaacggttaatttgcgtgatggacagactcttttactcggtggcctcactgattataaaaacacttctcaggattctggcgtaccgttcctgtctaaaatccctttaatcggcctcctgtttagctcccgctctgattctaacgaggaaagcacgttatacgtgctcgtcaaagcaaccatagtacgcgccctgtagcggcgcattaagcgcggcgggtgtggtggttacgcgcagcgtgaccgctacacttgccagcgccctagcgcccgctcctttcgctttcttcccttcctttctcgccacgttcgccggctttccccgtcaagctctaaatcgggggctccctttagggttccgatttagtgctttacggcacctcgaccccaaaaaacttgattagggtgatggttcacgtagtgggccatcgccctgatagacggtttttcgccctttgacgttggagtccacgttctttaatagtggactcttgttccaaactggaacaacactcaaccctatctcggtctattcttttgatttataagggattttgccgatttcggcctattggttaaaaaatgagctgatttaacaaaaatttaacgcgaattttaacaaaatattaacgtttacaatttaaatatttgcttatacaatcttcctgtttttggggcttttctgattatcaaccggggtacatatgattgacatgctagttttacgattaccgttcatcgattctcttgtttgctccagactctcaggcaatgacctgatagcctttgtagagacctctcaaaaatagctaccctctccggcatgaatttatcagctagaacggttgaatatcatattgatggtgatttgactgtctccggcctttctcacccgtttgaatctttacctacacattactcaggcattgcatttaaaatatatgagggttctaaaaatttttatccttgcgttgaaataaaggcttctcccgcaaaagtattacagggtcataatgtttttggtacaaccgatttagctttatgctctgaggctttattgcttaattttgctaattctttgccttgcctgtatgatttattggatgttggaattcctgatgcggtattttctccttacgcatctgtgcggtatttcacaccgcatatggtgcactctcagtacaatctgctctgatgccgcatagttaagccagccccgacacccgccaacacccgctgacgcgccctgacgggcttgtctgctcccggcatccgcttacagacaagctgtgaccgtctccgggagctgcatgtgtcagaggttttcaccgtcatcaccgaaacgcgcgagacgaaagggcctcgtgatacgcctatttttataggttaatgtcatgataataatggtttcttagacgtcaggtggcacttttcggggaaatgtgcgcggaacccctatttgtttatttttctaaatacattcaaatatgtatccgctcatgagacaataaccctgataaatgcttcaataatattgaaaaaggaagagtatgagtattcaacatttccgtgtcgcccttattcccttttttgcggcattttgccttcctgtttttgctcacccagaaacgctggtgaaagtaaaagatgctgaagatcagttgggtgcacgagtgggttacatcgaactggatctcaacagcggtaagatccttgagagttttcgccccgaagaacgttttccaatgatgagcacttttaaagttctgctatgtggcgcggtattatcccgtattgacgccgggcaagagcaactcggtcgccgcatacactattctcagaatgacttggttgagtactcaccagtcacagaaaagcatcttacggatggcatgacagtaagagaattatgcagtgctgccataaccatgagtgataacactgcggccaacttacttctgacaacgatcggaggaccgaaggagctaaccgcttttttgcacaacatgggggatcatgtaactcgccttgatcgttgggaaccggagctgaatgaagccataccaaacgacgagcgtgacaccacgatgcctgtagcaatggcaacaacgttgcgcaaactattaactggcgaactacttactctagcttcccggcaacaattaatagactggatggaggcggataaagttgcaggaccacttctgcgctcggcccttccggctggctggtttattgctgataaatctggagccggtgagcgtgggtctcgcggtatcattgcagcactggggccagatggtaagccctcccgtatcgtagttatctacacgacggggagtcaggcaactatggatgaacgaaatagacagatcgctgagataggtgcctcactgattaagcattggtaactgtcagaccaagtttactcatatatactttagattgatttaaaacttcatttttaatttaaaaggatctaggtgaagatcctttttgataatctcatgaccaaaatcccttaacgtgagttttcgttccactgagcgtcagaccccgtagaaaagatcaaaggatcttcttgagatcctttttttctgcgcgtaatctgctgcttgcaaacaaaaaaaccaccgctaccagcggtggtttgtttgccggatcaagagctaccaactctttttccgaaggtaactggcttcagcagagcgcagataccaaatactgtccttctagtgtagccgtagttaggccaccacttcaagaactctgtagcaccgcctacatacctcgctctgctaatcctgttaccagtggctgctgccagtggcgataagtcgtgtcttaccgggttggactcaagacgatagttaccggataaggcgcagcggtcgggctgaacggggggttcgtgcacacagcccagcttggagcgaacgacctacaccgaactgagatacctacagcgtgagctatgagaaagcgccacgcttcccgaagggagaaaggcggacaggtatccggtaagcggcagggtcggaacaggagagcgcacgagggagcttccagggggaaacgcctggtatctttatagtcctgtcgggtttcgccacctctgacttgagcgtcgatttttgtgatgctcgtcaggggggcggagcctatggaaaaacgccagcaacgcggcctttttacggttcctggccttttgctggccttttgctcacatgttctttcctgcgttatcccctgattctgtggataaccgtattaccgcctttgagtgagctgataccgctcgccgcagccgaacgaccgagcgcagcgagtcagtgagcgaggaagcggaagagcgcccaatacgcaaaccgcctctccccgcgcgttggccgattcattaatg

SEQ ID NO: 2 - DNA, 296 bp, Artificial Sequence
  Synthetic oligonucleotide
  misc_feature (1)..(8): FSE-I cut site
  misc_feature (9)..(136): miR-30 backbone
  misc_feature (139)..(160): miR-29c target (sense) strand
  misc_feature (161)..(175): miR-29c target (sense) strand
  misc_feature (176)..(199): miR-30 stem loop
  misc_feature (200)..(288): miR-29c guide (antisense) strand
  misc_feature (289)..(296): miR-30 backbone
ggccggcctgtttgaatgaggcttcagtactttacagaatcgttgcctgcacatcttggaaacacttgctgggattacttcttcaggttaacccaacagaaggctcgagaaggtatattgctgttgacagtgagcgcaaccgatttcaaatggtgctagagtgaagccacagatgtctagcaccatttgaaatcggttatgcctactgcctcggaattcaaggggctactttaggagcaattatcttgtttactaaaactgaataccttgctatctctttgatacattggccggcc

SEQ ID NO: 3 - DNA, 22 bp, Artificial Sequence
  Synthetic oligonucleotide
accgatttcaaatggtgctaga

SEQ ID NO: 4 - DNA, 24 bp, Artificial Sequence
  Synthetic oligonucleotide
tctagcaccatttgaaatcggtta

SEQ ID NO: 5 - DNA, 15 bp, Artificial Sequence
  Synthetic oligonucleotide
gtgaagccacagatg

SEQ ID NO: 6 - RNA, 98 nt, Artificial Sequence
  Synthetic oligonucleotide
  misc_feature (1)..(19): miR-30 backbone
  misc_feature (20)..(42): miR-29c target (sense) strand
  misc_feature (43)..(57): miR-30 stem loop
  misc_feature (58)..(81): miR-29c guide (antisense) strand
  misc_feature (82)..(98): miR-30 backbone
ugcuguugacagugagcgcaaccgauuucaaauggugcuagagugaagccacagaugucuagcaccauuugaaaucgguuaugccuacugccucggaa

SEQ ID NO: 7 - DNA, 3581 bp, Homo sapiens
  CDS (1)..(3579)
atgctgtggtgggaggaggtggaggattgttatgaaagggaggacgtgcagaagaagacttttaccaagtgggtgaacgctcagttcagcaaatttgggaagcagcacatcgagaatctgttttccgacctgcaggatgggagacggctgctggatctgctggaaggactgactggccagaagctgcccaaagagaaggggagcactagggtgcacgccctgaacaacgtgaacaaagctctgagagtgctgcagaacaacaacgtggatctggtgaatattggcagtactgatatcgtggacgggaaccacaaactgacactgggcctgatctggaacattattctgcactggcaggtgaaaaatgtgatgaagaacatcatggccgggctgcagcagaccaattccgagaagatcctgctgtcttgggtgcggcagagcacccgcaactatccccaggtgaacgtgattaacttcactacatcctggagcgacgggctggccctgaatgctctgattcacagccacaggcctgatctgttcgactggaatagcgtggtgtgccagcagtctgccacacagcgcctggaacatgccttcaatatcgctcggtaccagctggggatcgaaaaactgctggacccagaggatgtggacactacatacccagataaaaagtctattctgatgtacattactagcctgttccaggtgctgccacagcaggtgtctattgaagccattcaggaggtggaaatgctgccccgcccccccaaagtgactaaagaggagcattttcagctgcatcatcagatgcattacagccagcagattaccgtgagcctggctcagggatatgagcgcaccagtagtccaaaaccacggttcaagtcctacgcttatacccaggctgcctacgtgacaactagcgaccctactagatccccctttccatcccagcacctggaggccccagaggacaagagctttgggtccagcctgatggaaagcgaggtgaatctggatcggtaccagacagccctggaggaggtgctgagctggctgctgagtgctgaagacacactgcaggcccagggcgaaatttccaatgacgtggaagtggtgaaggatcagttccacacacacgagggctatatgatggacctgacagctcaccaggggcgcgtgggcaatatcctgcagctgggctctaaactgatcggcaccgggaaactgagtgaggacgaggaaacagaagtgcaggagcagatgaacctgctgaacagccgctgggagtgtctgagagtggctagtatggagaagcagtccaacctgcaccgggtgctgatggacctgcagaaccagaaactgaaagagctgaacgactggctgacaaagactgaggaacgcacaaggaagatggaggaggagccactgggacccgacctggaggatctgaagagacaggtgcagcagcataaggtgctgcaggaggatctggaacaggagcaggtgcgggtgaactccctgacacatatggtggtggtggtggacgaatctagtggagatcacgccaccgccgccctggaggaacagctgaaggtgctgggggaccggtgggccaacatttgccggtggaccgaggacaggtgggtgctgctgcaggacatcctgctgaaatggcagaggctgaccgaggagcagtgtctgtttagtgcttggctgagcgagaaagaggacgccgtgaacaagatccacacaaccggctttaaggatcagaacgaaatgctgtctagcctgcagaaactggctgtgctgaaggccgatctggagaaaaagaagcagagcatgggcaaactgtatagcctgaaacaggacctgctgagcaccctgaagaacaagagcgtgacccagaagacagaagcctggctggataactttgcccgctgctgggacaacctggtgcagaaactggagaaaagtacagctcagatctctcaggctgtgaccacaacccagcctagcctgacccagacaaccgtgatggaaaccgtgaccaccgtgacaacccgcgaacagatcctggtgaaacatgcccaggaagagctgccacctccacctccccagaagaagagaaccctggagcggctgcaggagctgcaggaagccactgacgaactggacctgaagctgaggcaggccgaagtgattaaggggtcttggcagcctgtgggcgatctgctgattgattccctgcaggaccacctggaaaaggtgaaggctctgagaggcgaaattgctccactgaaggagaacgtgagtcatgtgaacgatctggctagacagctgacaacactgggcatccagctgagcccatacaatctgagcacactggaggacctgaataccaggtggaagctgctgcaggtggctgtggaagaccgggtgcggcagctgcatgaggcccatcgcgacttcggaccagccagccagcactttctgagcacatccgtgcaggggccctgggagagggccatttctcccaacaaggtgccctactatattaatcacgagacccagaccacttgttgggaccatcccaagatgacagaactgtaccagtccctggccgatctgaacaacgtgaggtttagcgcttacagaaccgctatgaagctgagacggctgcagaaggccctgtgcctggatctgctgtccctgtccgccgcctgcgatgccctggatcagcataatctgaagcagaacgatcagccaatggatatcctgcagatcatcaactgcctgaccactatctacgacaggctggagcaggagcacaacaacctggtgaacgtgcctctgtgcgtggatatgtgcctgaactggctgctgaacgtgtatgacactgggcgcaccggccggatcagagtgctgagttttaaaactgggattatctccctgtgtaaggcccacctggaggacaagtacaggtacctgttcaagcaggtggctagtagcactggattttgtgaccagcgccgcctgggactgctgctgcatgatagtatccagattcctagacagctgggagaggtggctagtttcggaggatctaacatcgaacccagcgtgcgcagctgtttccagtttgccaataacaaacctgaaatcgaggctgctctgttcctggattggatgcgcctggaaccacagagcatggtgtggctgcctgtgctgcacagagtggctgccgccgaaactgccaagcaccaggctaaatgcaacatctgcaaggaatgtcccattatcggctttcgctacaggagtctgaaacattttaactacgatatttgccagagctgcttcttttccggaagagtggccaaaggacacaagatgcactaccctatggtggaatattgcaccccaactacatctggcgaagatgtgcgcgattttgccaaggtgctgaagaataagtttcggactaagaggtacttcgccaagcacccccgcatggggtatctgccagtgcagacagtgctggaaggagacaatatggagaccgatacaatgtgagc

SEQ ID NO: 8 - protein, 1192 aa, Homo sapiens
MLWWEEVEDCYEREDVQKKTFTKWVNAQFSKFGKQHIENLFSDLQDGRRLLDLLEGLTGQKLPKEKGSTRVHALNNVNKALRVLQNNNVDLVNIGSTDIVDGNHKLTLGLIWNIILHWQVKNVMKNIMAGLQQTNSEKILLSWVRQSTRNYPQVNVINFTTSWSDGLALNALIHSHRPDLFDWNSVVCQQSATQRLEHAFNIARYQLGIEKLLDPEDVDTTYPDKKSILMYITSLFQVLPQQVSIEAIQEVEMLPRPPKVTKEEHFQLHHQMHYSQQITVSLAQGYERTSSPKPRFKSYAYTQAAYVTTSDPTRSPFPSQHLEAPEDKSFGSSLMESEVNLDRYQTALEEVLSWLLSAEDTLQAQGEISNDVEVVKDQFHTHEGYMMDLTAHQGRVGNILQLGSKLIGTGKLSEDEETEVQEQMNLLNSRWECLRVASMEKQSNLHRVLMDLQNQKLKELNDWLTKTEERTRKMEEEPLGPDLEDLKRQVQQHKVLQEDLEQEQVRVNSLTHMVVVVDESSGDHATAALEEQLKVLGDRWANICRWTEDRWVLLQDILLKWQRLTEEQCLFSAWLSEKEDAVNKIHTTGFKDQNEMLSSLQKLAVLKADLEKKKQSMGKLYSLKQDLLSTLKNKSVTQKTEAWLDNFARCWDNLVQKLEKSTAQISQAVTTTQPSLTQTTVMETVTTVTTREQILVKHAQEELPPPPPQKKRTLERLQELQEATDELDLKLRQAEVIKGSWQPVGDLLIDSLQDHLEKVKALRGEIAPLKENVSHVNDLARQLTTLGIQLSPYNLSTLEDLNTRWKLLQVAVEDRVRQLHEAHRDFGPASQHFLSTSVQGPWERAISPNKVPYYINHETQTTCWDHPKMTELYQSLADLNNVRFSAYRTAMKLRRLQKALCLDLLSLSAACDALDQHNLKQNDQPMDILQIINCLTTIYDRLEQEHNNLVNVPLCVDMCLNWLLNVYDTGRTGRIRVLSFKTGIISLCKAHLEDKYRYLFKQVASSTGFCDQRRLGLLLHDSIQIPRQLGEVASFGGSNIEPSVRSCFQFANNKPEIEAALFLDWMRLEPQSMVWLPVLHRVAAAETAKHQAKCNICKECPIIGFRYRSLKHFNYDICQSCFFSGRVAKGHKMHYPMVEYCTPTTSGEDVRDFAKVLKNKFRTKRYFAKHPRMGYLPVQTVLEGDNMETDTM

SEQ ID NO: 9 - DNA, 8409 bp, Adeno-associated virus
  promoter (236)..(799): MCK promotor
  Intron (844)..(993): Chimeric intron sequence
  misc_feature (1004)..(4584): Human Dystrophin sequence
  misc_feature (4585)..(4640): Poly A tail
  misc_feature (6606)..(7466): Ampicillin resistance
  misc_feature (7621)..(8240): pGEX plasmid backbone with pBR322 origin or replication
gcccaatacgcaaaccgcctctccccgcgcgttggccgattcattaatgcagctggcgcgctcgctcgctcactgaggccgcccgggcaaagcccgggcgtcgggcgacctttggtcgcccggcctcagtgagcgagcgagcgcgcagagagggagtggccaactccatcactaggggttccttgtagttaatgattaacccgccatgctaattatctacgtagccatgtctagacagccactatgggtctaggctgcccatgtaaggaggcaaggcctggggacacccgagatgcctggttataattaacccagacatgtggctgctccccccccccaacacctgctgcctgagcctcacccccaccccggtgcctgggtcttaggctctgtacaccatggaggagaagctcgctctaaaaataaccctgtccctggtgggctgtgggggactgagggcaggctgtaacaggcttgggggccagggcttatacgtgcctgggactcccaaagtattactgttccatgttcccggcgaagggccagctgtcccccgccagctagactcagcacttagtttaggaaccagtgagcaagtcagcccttggggcagcccatacaaggccatggggctgggcaagctgcacgcctgggtccggggtgggcacggtgcccgggcaacgagctgaaagctcatctgctctcaggggcccctccctggggacagcccctcctggctagtcacaccctgtaggctcctctatataacccaggggcacaggggctgcccccgggtcaccaccacctccacagcacagacagacactcaggagccagccagccaggtaagtttagtctttttgtcttttatttcaggtcccggatccggtggtggtgcaaatcaaagaactgctcctcagtggatgttgcctttacttctaggcctgtacggaagtgttacttctgctctaaaagctgcggaattgtacccgcggccgccaccatgctgtggtgggaggaggtggaggattgttatgaaagggaggacgtgcagaagaagacttttaccaagtgggtgaacgctcagttcagcaaatttgggaagcagcacatcgagaatctgttttccgacctgcaggatgggagacggctgctggatctgctggaaggactgactggccagaagctgcccaaagagaaggggagcactagggtgcacgccctgaacaacgtgaacaaagctctgagagtgctgcagaacaacaacgtggatctggtgaatattggcagtactgatatcgtggacgggaaccacaaactgacactgggcctgatctggaacattattctgcactggcaggtgaaaaatgtgatgaagaacatcatggccgggctgcagcagaccaattccgagaagatcctgctgtcttgggtgcggcagagcacccgcaactatccccaggtgaacgtgattaacttcactacatcctggagcgacgggctggccctgaatgctctgattcacagccacaggcctgatctgttcgactggaatagcgtggtgtgccagcagtctgccacacagcgcctggaacatgccttcaatatcgctcggtaccagctggggatcgaaaaactgctggacccagaggatgtggacactacatacccagataaaaagtctattctgatgtacattactagcctgttccaggtgctgccacagcaggtgtctattgaagccattcaggaggtggaaatgctgccccgcccccccaaagtgactaaagaggagcattttcagctgcatcatcagatgcattacagccagcagattaccgtgagcctggctcagggatatgagcgcaccagtagtccaaaaccacggttcaagtcctacgcttatacccaggctgcctacgtgacaactagcgaccctactagatccccctttccatcccagcacctggaggccccagaggacaagagctttgggtccagcctgatggaaagcgaggtgaatctggatcggtaccagacagccctggaggaggtgctgagctggctgctgagtgctgaagacacactgcaggcccagggcgaaatttccaatgacgtggaagtggtgaaggatcagttccacacacacgagggctatatgatggacctgacagctcaccaggggcgcgtgggcaatatcctgcagctgggctctaaactgatcggcaccgggaaactgagtgaggacgaggaaacagaagtgcaggagcagatgaacctgctgaacagccgctgggagtgtctgagagtggctagtatggagaagcagtccaacctgcaccgggtgctgatggacctgcagaaccagaaactgaaagagctgaacgactggctgacaaagactgaggaacgcacaaggaagatggaggaggagccactgggacccgacctggaggatctgaagagacaggtgcagcagcataaggtgctgcaggaggatctggaacaggagcaggtgcgggtgaactccctgacacatatggtggtggtggtggacgaatctagtggagatcacgccaccgccgccctggaggaacagctgaaggtgctgggggaccggtgggccaacatttgccggtggaccgaggacaggtgggtgctgctgcaggacatcctgctgaaatggcagaggctgaccgaggagcagtgtctgtttagtgcttggctgagcgagaaagaggacgccgtgaacaagatccacacaaccggctttaaggatcagaacgaaatgctgtctagcctgcagaaactggctgtgctgaaggccgatctggagaaaaagaagcagagcatgggcaaactgtatagcctgaaacaggacctgctgagcaccctgaagaacaagagcgtgacccagaagacagaagcctggctggataactttgcccgctgctgggacaacctggtgcagaaactggagaaaagtacagctcagatctctcaggctgtgaccacaacccagcctagcctgacccagacaaccgtgatggaaaccgtgaccaccgtgacaacccgcgaacagatcctggtgaaacatgcccaggaagagctgccacctccacctccccagaagaagagaaccctggagcggctgcaggagctgcaggaagccactgacgaactggacctgaagctgaggcaggccgaagtgattaaggggtcttggcagcctgtgggcgatctgctgattgattccctgcaggaccacctggaaaaggtgaaggctctgagaggcgaaattgctccactgaaggagaacgtgagtcatgtgaacgatctggctagacagctgacaacactgggcatccagctgagcccatacaatctgagcacactggaggacctgaataccaggtggaagctgctgcaggtggctgtggaagaccgggtgcggcagctgcatgaggcccatcgcgacttcggaccagccagccagcactttctgagcacatccgtgcaggggccctgggagagggccatttctcccaacaaggtgccctactatattaatcacgagacccagaccacttgttgggaccatcccaagatgacagaactgtaccagtccctggccgatctgaacaacgtgaggtttagcgcttacagaaccgctatgaagctgagacggctgcagaaggccctgtgcctggatctgctgtccctgtccgccgcctgcgatgccctggatcagcataatctgaagcagaacgatcagccaatggatatcctgcagatcatcaactgcctgaccactatctacgacaggctggagcaggagcacaacaacctggtgaacgtgcctctgtgcgtggatatgtgcctgaactggctgctgaacgtgtatgacactgggcgcaccggccggatcagagtgctgagttttaaaactgggattatctccctgtgtaaggcccacctggaggacaagtacaggtacctgttcaagcaggtggctagtagcactggattttgtgaccagcgccgcctgggactgctgctgcatgatagtatccagattcctagacagctgggagaggtggctagtttcggaggatctaacatcgaacccagcgtgcgcagctgtttccagtttgccaataacaaacctgaaatcgaggctgctctgttcctggattggatgcgcctggaaccacagagcatggtgtggctgcctgtgctgcacagagtggctgccgccgaaactgccaagcaccaggctaaatgcaacatctgcaaggaatgtcccattatcggctttcgctacaggagtctgaaacattttaactacgatatttgccagagctgcttcttttccggaagagtggccaaaggacacaagatgcactaccctatggtggaatattgcaccccaactacatctggcgaagatgtgcgcgattttgccaaggtgctgaagaataagtttcggactaagaggtacttcgccaagcacccccgcatggggtatctgccagtgcagacagtgctggaaggagacaatatggagaccgatacaatgtgagcggccgcaataaaagatctttattttcattagatctgtgtgttggttttttgtgtgtctagagcatggctacgtagataagtagcatggcgggttaatcattaactacaaggaacccctagtgatggagttggccactccctctctgcgcgctcgctcgctcactgaggccgggcgaccaaaggtcgcccgacgcccgggctttgcccgggcggcctcagtgagcgagcgagcgcgccagctggcgtaatagcgaagaggcccgcaccgatcgcccttcccaacagttgcgcagcctgaatggcgaatggaagttccagacgattgagcgtcaaaatgtaggtatttccatgagcgtttttcctgttgcaatggctggcggtaatattgttctggatattaccagcaaggccgatagtttgagttcttctactcaggcaagtgatgttattactaatcaaagaagtattgcgacaacggttaatttgcgtgatggacagactcttttactcggtggcctcactgattataaaaacacttctcaggattctggcgtaccgttcctgtctaaaatccctttaatcggcctcctgtttagctcccgctctgattctaacgaggaaagcacgttatacgtgctcgtcaaagcaaccatagtacgcgccctgtagcggcgcattaagcgcggcgggtgtggtggttacgcgcagcgtgaccgctacacttgccagcgccctagcgcccgctcctttcgctttcttcccttcctttctcgccacgttcgccggctttccccgtcaagctctaaatcgggggctccctttagggttccgatttagtgatttacggcacctcgaccccaaaaaacttgattagggtgatggttcacgtagtgggccatcgccctgatagacggtttttcgccctttgacgttggagtccacgttctttaatagtggactcttgttccaaactggaacaacactcaaccctatctcggtctattcttttgatttataagggattttgccgatttcggcctattggttaaaaaatgagctgatttaacaaaaatttaacgcgaattttaacaaaatattaacgtttacaatttaaatatttgcttatacaatcttcctgtttttggggcttttctgattatcaaccggggtacatatgattgacatgctagttttacgattaccgttcatcgattctcttgtttgctccagactctcaggcaatgacctgatagcctttgtagagacctctcaaaaatagctaccctctccggcatgaatttatcagctagaacggttgaatatcatattgatggtgatttgactgtctccggcctttctcacccgtttgaatctttacctacacattactcaggcattgcatttaaaatatatgagggttctaaaaatttttatccttgcgttgaaataaaggcttctcccgcaaaagtattacagggtcataatgtttttggtacaaccgatttagctttatgctctgaggctttattgcttaattttgctaattctttgccttgcctgtatgatttattggatgttggaagttcctgatgcggtattttctccttacgcatctgtgcggtatttcacaccgcatatggtgcactctcagtacaatctgctctgatgccgcatagttaagccagccccgacacccgccaacacccgctgacgcgccctgacgggcttgtctgctcccggcatccgcttacagacaagctgtgaccgtctccgggagctgcatgtgtcagaggttttcaccgtcatcaccgaaacgcgcgagacgaaagggcctcgtgatacgcctatttttataggttaatgtcatgataataatggtttcttagacgtcaggtggcacttttcggggaaatgtgcgcggaacccctatttgtttatttttctaaatacattcaaatatgtatccgctcatgagacaataaccctgataaatgcttcaataatattgaaaaaggaagagtatgagtattcaacatttccgtgtcgcccttattcccttttttgcggcattttgccttcctgtttttgctcacccagaaacgctggtgaaagtaaaagatgctgaagatcagttgggtgcacgagtgggttacatcgaactggatctcaacagcggtaagatccttgagagttttcgccccgaagaacgttttccaatgatgagcacttttaaagttctgctatgtggcgcggtattatcccgtattgacgccgggcaagagcaactcggtcgccgcatacactattctcagaatgacttggttgagtactcaccagtcacagaaaagcatcttacggatggcatgacagtaagagaattatgcagtgctgccataaccatgagtgataacactgcggccaacttacttctgacaacgatcggaggaccgaaggagctaaccgcttttttgcacaacatgggggatcatgtaactcgccttgatcgttgggaaccggagctgaatgaagccataccaaacgacgagcgtgacaccacgatgcctgtagcaatggcaacaacgttgcgcaaactattaactggcgaactacttactctagcttcccggcaacaattaatagactggatggaggcggataaagttgcaggaccacttctgcgctcggcccttccggctggctggtttattgctgataaatctggagccggtgagcgtgggtctcgcggtatcattgcagcactggggccagatggtaagccctcccgtatcgtagttatctacacgacggggagtcaggcaactatggatgaacgaaatagacagatcgctgagataggtgcctcactgattaagcattggtaactgtcagaccaagtttactcatatatactttagattgatttaaaacttcatttttaatttaaaaggatctaggtgaagatcctttttgataatctcatgaccaaaatcccttaacgtgagttttcgttccactgagcgtcagaccccgtagaaaagatcaaaggatcttcttgagatcctttttttctgcgcgtaatctgctgcttgcaaacaaaaaaaccaccgctaccagcggtggtttgtttgccggatcaagagctaccaactctttttccgaaggtaactggcttcagcagagcgcagataccaaatactgtccttctagtgtagccgtagttaggccaccacttcaagaactctgtagcaccgcgtacatacctcgctctgctaatcctgttaccagtggctgctgccagtggcgataagtcgtgtcttaccgggttggactcaagacgatagttaccggataaggcgcagcggtcgggctgaacggggggttcgtgcacacagcccagcttggagcgaacgacctacaccgaactgagatacctacagcgtgagctatgagaaagcgccacgcttcccgaagggagaaaggcggacaggtatccggtaagcggcagggtcggaacaggagagcgcacgagggagcttccagggggaaacgcctggtatctttatagtcctgtcgggtttcgccacctctgacttgagcgtcgatttttgtgatgctcgtcaggggggcggagcctatggaaaaacgccagcaacgcggcctttttacggttcctggccttttgctggccttttgctcacatgttctttcctgcgttatcccctgattctgtggataaccgtattaccgggtttgagtgagctgataccgctcgccgcagccgaacgaccgagcgcagcgagtcagtgagcgaccaagcggaagagc

SEQ ID NO: 10 - DNA, 206 bp, Artificial Sequence
  Synthetic oligonucleotide
  enhancer (1)..(206): MCK enhancer
cagccactatgggtctaggctgcccatgtaaggaggcaaggcctggggacacccgagatgcctggttataattaacccagacatgtggctgctccccccccccaacacctgctgcctgagcctcacccccaccccggtgcctgggtcttaggctctgtacaccatggaggagaagctcgctctaaaaataaccctgtccctggtgg

SEQ ID NO: 11 - DNA, 358 bp, Artificial Sequence
  Synthetic oligonucleotide
  promoter (1)..(358): MCK promoter
gctgtgggggactgagggcaggctgtaacaggcttgggggccagggcttatacgtgcctgggactcccaaagtattactgttccatgttcccggcgaagggccagctgtcccccgccagctagactcagcacttagtttaggaaccagtgagcaagtcagcccttggggcagcccatacaaggccatggggctgggcaagctgcacgcctgggtccggggtgggcacggtgcccgggcaacgagctgaaagctcatctgctctcaggggcccctccctggggacagcccctcctggctagtcacaccctgtaggctcctctatataacccaggggcacaggggctgcccccgggtcac

SEQ ID NO: 12 - DNA, 5920 bp, Adeno-associated virus
  misc_feature: pAAV.MCK.miR26C Sequence
  misc_feature (4)..(9): n is a, c, g, t or u
  enhancer (190)..(395): MCK enhancer
  promoter (396)..(753): MCK promoter
  misc_feature (1316)..(1608): shRNA-miR29-c with primary seed sequence
  misc_feature (1487)..(1512): miR-29c
  misc_feature (2094)..(2146): SV40 PolyA
  misc_feature (2326)..(2331): n is a, c, g, t or u
ctgnnnnnngcgcgctcgctcgctcactgaggccgcccgggcaaagcccgggcgtcgggcgacctttggtcgcccggcctcagtgagcgagcgagcgcgcagagagggagtggccaactccatcactaggggttccttgtagttaatgattaacccgccatgctaattatctacgtagccatgtctagacagccactatgggtctaggctgcccatgtaaggaggcaaggcctggggacacccgagatgcctggttataattaacccagacatgtggctgctccccccccccaacacctgctgcctgagcctcacccccaccccggtgcctgggtcttaggctctgtacaccatggaggagaagctcgctctaaaaataaccctgtccctggtgggctgtgggggactgagggcaggctgtaacaggcttgggggccagggcttatacgtgcctgggactcccaaagtattactgttccatgttcccggcgaagggccagctgtcccccgccagctagactcagcacttagtttaggaaccagtgagcaagtcagcccttggggcagcccatacaaggccatggggctgggcaagctgcacgcctgggtccggggtgggcacggtgcccgggcaacgagctgaaagctcatctgctctcaggggcccctccctggggacagcccctcctggctagtcacaccctgtaggctcctctatataacccaggggcacaggggctgcccccgggtcaccaccacctccacagcacagacagacactcaggagccagccagccaggtaagtttagtctttttgtcttttatttcaggtcccggatccggtggtggtgcaaatcaaagaactgctcctcagtggatgttgcctttacttctaggcctgtacggaagtgttacttctgctctaaaagctgcggaattgtacccgcctagaggatccggtactcgaggaactgaaaaaccagaaagttaactggtaagtttagtctttttgtcttttatttcaggtcccggatccggtggtggtgcaaatcaaagaactgctcctcagtggatgttgcctttacttctaggcctgtacggaagtgttacttctgctctaaaagctgcggaattgtacccggggccgatccaccggtctttttcgcaacgggtttgccgccagaacacaggtaagtgccgtgtgtggttcccgcgggcggcgacggggcccgtgcgtcccagcgcacatgttcggcgaggcggggcctgcgagcgcggccaccgagaatcggacgggggtagtctcaagctggccggcctgtttgaatgaggcttcagtactttacagaatcgttgcctgcacatcttggaaacacttgctgggattacttcttcaggttaacccaacagaaggctcgagaaggtatattgctgttgacagtgagcgcaaccgatttcaaatggtgctagagtgaagccacagatgtctagcaccatttgaaatcggttatgcctactgcctcggaattcaaggggctactttaggagcaattatcttgtttactaaaactgaataccttgctatctctttgatacattggccggcctgctctggtgcctggcctcgcgccgccgtgtatcgccccgccctgggcggcaaggctggcccggtcggcaccagttgcgtgagcggaaagatggccgcttcccggccctgctgcagggagctcaaaatggaggacgcggcgctcgggagagcgggcgggtgagtcacccacacaaaggaaaagggcctttccgtcctcagccgtcgcttcatgtgactccacggagtaccgggcgccgtccaggcacctcgattagttctcgagcttttggagtacgtcgtctttaggttggggggaggggttttatgcgatggagtttccccacactgagtgggtggagactgaagttaggccagcttggcacttgatgtaattctccttggaatttgccctttttgagtttggatcttggttcattctcaagcctcagacagtggttcaaagtttttttcttccatttcaggtgtcgtgaaaagctagtgcggccgcaataaaagatctttattttcattagatctgtgtgttggttttttgtgtgtctagacatggctacgtagataattagcatggcgggttaatcattaactacaaggaacccctagtgatggagttggccactccctctctgcgcgctcgctcgctcactgaggccgggcgaccaaaggtcgcccgacgcccgggctttgcccgggcggcctcagtgagcgagcgagcgcgcnnnnnncagctggcgtaatagcgaagaggcccgcaccgatcgcccttcccaacagttgcgcagcctgaatggcgaatggaagttccagacgattgagcgtcaaaatgtaggtatttccatgagcgtttttcctgttgcaatggctggcggtaatattgttctggatattaccagcaaggccgatagtttgagttcttctactcaggcaagtgatgttattactaatcaaagaagtattgcgacaacggttaatttgcgtgatggacagactcttttactcggtggcctcactgattataaaaacacttctcaggattctggcgtaccgttcctgtctaaaatccctttaatcggcctcctgtttagctcccgctctgattctaacgaggaaagcacgttatacgtgctcgtcaaagcaaccatagtacgcgccctgtagcggcgcattaagcgcggcgggtgtggtggttacgcgcagcgtgaccgctacacttgccagcgccctagcgcccgctcctttcgctttcttcccttcctttctcgccacgttcgccggctttccccgtcaagctctaaatcgggggctccctttagggttccgatttagtgatttacggcacctcgaccccaaaaaacttgattagggtgatggttcacgtagtgggccatcgccctgatagacggtttttcgccctttgacgttggagtccacgttctttaatagtggactcttgttccaaactggaacaacactcaaccctatctcggtctattcttttgatttataagggattttgccgatttcggcctattggttaaaaaatgagctgatttaacaaaaatttaacgcgaattttaacaaaatattaacgtttacaatttaaatatttgcttatacaatcttcctgtttttggggcttttctgattatcaaccggggtacatatgattgacatgctagttttacgattaccgttcatcgattctcttgtttgctccagactctcaggcaatgacctgatagcctttgtagagacctctcaaaaatagctaccctctccggcatgaatttatcagctagaacggttgaatatcatattgatggtgatttgactgtctccggcctttctcacccgtttgaatctttacctacacattactcaggcattgcatttaaaatatatgagggttctaaaaatttttatccttgcgttgaaataaaggcttctcccgcaaaagtattacagggtcataatgtttttggtacaaccgatttagctttatgctctgaggctttattgcttaattttgctaattctttgccttgcctgtatgatttattggatgttggaagttcctgatgcggtattttctccttacgcatctgtgcggtatttcacaccgcatatggtgcactctcagtacaatctgctctgatgccgcatagttaagccagccccgacacccgccaacacccgctgacgcgccctgacgggcttgtctgctcccggcatccgcttacagacaagctgtgaccgtctccgggagctgcatgtgtcagaggttttcaccgtcatcaccgaaacgcgcgagacgaaagggcctcgtgatacgcctatttttataggttaatgtcatgataataatggtttcttagacgtcaggtggcacttttcggggaaatgtgcgcggaacccctatttgtttatttttctaaatacattcaaatatgtatccgctcatgagacaataaccctgataaatgcttcaataatattgaaaaaggaagagtatgagtattcaacatttccgtgtcgcccttattcccttttttgcggcattttgccttcctgtttttgctcacccagaaacgctggtgaaagtaaaagatgctgaagatcagttgggtgcacgagtgggttacatcgaactggatctcaacagcggtaagatccttgagagttttcgccccgaagaacgttttccaatgatgagcacttttaaagttctgctatgtggcgcggtattatcccgtattgacgccgggcaagagcaactcggtcgccgcatacactattctcagaatgacttggttgagtactcaccagtcacagaaaagcatcttacggatggcatgacagtaagagaattatgcagtgctgccataaccatgagtgataacactgcggccaacttacttctgacaacgatcggaggaccgaaggagctaaccgcttttttgcacaacatgggggatcatgtaactcgccttgatcgttgggaaccggagctgaatgaagccataccaaacgacgagcgtgacaccacgatgcctgtagcaatggcaacaacgttgcgcaaactattaactggcgaactacttactctagcttcccggcaacaattaatagactggatggaggcggataaagttgcaggaccacttctgcgctcggcccttccggctggctggtttattgctgataaatctggagccggtgagcgtgggtctcgcggtatcattgcagcactggggccagatggtaagccctcccgtatcgtagttatctacacgacggggagtcaggcaactatggatgaacgaaatagacagatcgctgagataggtgcctcactgattaagcattggtaactgtcagaccaagtttactcatatatactttagattgatttaaaacttcatttttaatttaaaaggatctaggtgaagatcctttttgataatctcatgaccaaaatcccttaacgtgagttttcgttccactgagcgtcagaccccgtagaaaagatcaaaggatcttcttgagatcctttttttctgcgcgtaatctgctgcttgcaaacaaaaaaaccaccgctaccagcggtggtttgtttgccggatcaagagctaccaactctttttccgaaggtaactggcttcagcagagcgcagataccaaatactgtccttctagtgtagccgtagttaggccaccacttcaagaactctgtagcaccgcgtacatacctcgctctgctaatcctgttaccagtggctgctgccagtggcgataagtcgtgtcttaccgggttggactcaagacgatagttaccggataaggcgcagcggtcgggctgaacggggggttcgtgcacacagcccagcttggagcgaacgacctacaccgaactgagatacctacagcgtgagctatgagaaagcgccacgcttcccgaagggagaaaggcggacaggtatccggtaagcggcagggtcggaacaggagagcgcacgagggagcttccagggggaaacgcctggtatctttatagtcctgtcgggtttcgccacctctgacttgagcgtcgatttttgtgatgctcgtcaggggggcggagcctatggaaaaacgccagcaacgcggcctttttacggttcctggccttttgctggccttttgctcacatgttctttcctgcgttatcccctgattctgtggataaccgtattaccgggtttgagtgagctgataccgctcgccgcagccgaacgaccgagcgcagcgagtcagtgagcgaccaagcggaagagc